European Patent Specification EP 3 515 938 B1, published January 8, 2025. Title: The novel monoclonal antibodies to programmed death 1 (PD-1). Applicant: WuXi Biologics (Shanghai) Co., Ltd. The sequence listing filed with the application follows.

SEQUENCE LISTING (24 sequences)

SEQ ID NO: 1 - protein, 115 aa, Artificial Sequence
QVQLVQSGAEVKKPGSSVKVSCKASGFTFTTYYISWVRQAPGQGLEYLGYINMGSGGTNYNEKFKGRVTITADKSTSTAYMELSSLRSEDTAVYYCAILGYFDYWGQGTMVTVSS

SEQ ID NO: 2 - protein, 115 aa, Artificial Sequence
QVQLVQSGAEVKKPGSSVKVSCKASGFTFTTYYISWVRQAPGQGLEYLGYINMGSGGTNYNEKFKGRVTITADKSTSTAYMELSSLRSEDTAVYYCAIIGYFDYWGQGTMVTVSS

SEQ ID NO: 3 - protein, 112 aa, Artificial Sequence
DVVMTQSPLSLPVTLGQPASISCRSSQSLLDSDGGTYLYWFQQRPGQSPRRLIYLVSTLGSGVPDRFSGSGSGTDFTLKISRVEAEDVGVYYCMQLTHWPYTFGQGTKLEIK

SEQ ID NO: 4 - protein, 112 aa, Artificial Sequence
DVVMTQSPLSLPVTLGQPASISCRSSQSLLDSDGSTYLYWFQQRPGQSPRRLIYLVSTLGSGVPDRFSGSGSGTDFTLKISRVEAEDVGVYYCMQLTHWPYTFGQGTKLEIK

SEQ ID NO: 5 - protein, 112 aa, Artificial Sequence
DVVMTQSPLSLPVTLGQPASISCRSSQSLLDSDGATYLYWFQQRPGQSPRRLIYLVSTLGSGVPDRFSGSGSGTDFTLKISRVEAEDVGVYYCMQLTHWPYTFGQGTKLEIK

SEQ ID NO: 6 - protein, 112 aa, Artificial Sequence
DVVMTQSPLSLPVTLGQPASISCRSSQSLLDSDGNTYLYWFQQRPGQSPRRLIYLVSTLGSGVPDRFSGSGSGTDFTLKISRVEAEDVGVYYCMQLTHWPYTFGQGTKLEIK

SEQ ID NO: 7 - protein, 112 aa, Artificial Sequence
DVVMTQSPLSLPVTLGQPASISCRSSQSLLDSDGNTYLYWFQQRPGQSPRRLIYLVSTLGSGVPDRFSGSGSGTDFTLKISRVEAEDVGVYYCMQLTHAPYTFGQGTKLEIK

SEQ ID NO: 8 - protein, 112 aa, Artificial Sequence
DVVMTQSPLSLPVTLGQPASISCRSSQSLLDSDGQTYLYWFQQRPGQSPRRLIYLVSTLGSGVPDRFSGSGSGTDFTLKISRVEAEDVGVYYCMQLTHEPYTFGQGTKLEIK

SEQ ID NO: 9 - protein, 112 aa, Artificial Sequence
DVVMTQSPLSLPVTLGQPASISCRSSQSLLDSDGQTYLYWFQQRPGQSPRRLIYLVSTLGSGVPDRFSGSGSGTDFTLKISRVEAEDVGVYYCMQLTHENYTFGQGTKLEIK

SEQ ID NO: 10 - protein, 5 aa, Artificial Sequence
TYYIS

SEQ ID NO: 11 - protein, 17 aa, Artificial Sequence
YINMGSGGTNYNEKFKG

SEQ ID NO: 12 - protein, 6 aa, Artificial Sequence
LGYFDY

SEQ ID NO: 13 - protein, 6 aa, Artificial Sequence
IGYFDY

SEQ ID NO: 14 - protein, 16 aa, Artificial Sequence
RSSQSLLDSDGGTYLY

SEQ ID NO: 15 - protein, 16 aa, Artificial Sequence
RSSQSLLDSDGSTYLY

SEQ ID NO: 16 - protein, 16 aa, Artificial Sequence
RSSQSLLDSDGATYLY

SEQ ID NO: 17 - protein, 16 aa, Artificial Sequence
RSSQSLLDSDGNTYLY

SEQ ID NO: 18 - protein, 16 aa, Artificial Sequence
RSSQSLLDSDGQTYLY

SEQ ID NO: 19 - protein, 7 aa, Artificial Sequence
LVSTLGS

SEQ ID NO: 20 - protein, 9 aa, Artificial Sequence
MQLTHENYT

SEQ ID NO: 21 - protein, 9 aa, Artificial Sequence
MQLTHWPYT

SEQ ID NO: 22 - protein, 9 aa, Artificial Sequence
MQLTHAPYT

SEQ ID NO: 23 - protein, 9 aa, Artificial Sequence
MQLTHEPYT

SEQ ID NO: 24 - protein, 288 aa, homo sapiens
MQIPQAPWPVVWAVLQLGWRPGWFLDSPDRPWNPPTFSPALLVVTEGDNATFTCSFSNTSESFVLNWYRMSPSNQTDKLAAFPEDRSQPGQDCRFRVTQLPNGRDFHMSVVRARRNDSGTYLCGAISLAPKAQIKESLRAELRVTERRAEVPTAHPSPSPRPAGQFQTLVVGVVGGLLGSLVLLVWVLAVICSRAARGTIGARRTGQPLKEDPSAVPVFSVDYGELDFQWREKTPEPPVPCVPEQTEYATIVFPSGMGTSSPARRGSADGPRSAQPLRPEDGHCSWPL